European Patent Application EP 4 487 700 A1, published January 8, 2025. Title: EGG WHITE PROTEIN ANTI-INFLAMMATORY PEPTIDE AND APPLICATION THEREOF. Applicant: Hangzhou BIBAU Biotechnology Co., Ltd. Application US. The sequence listing filed with the application follows.

SEQUENCE LISTING (9 sequences)

SEQ ID NO: 1 - protein, 4 aa, unidentified
FGPH

SEQ ID NO: 2 - protein, 7 aa, unidentified
WNIPIGT

SEQ ID NO: 3 - protein, 9 aa, unidentified
AGWNIPIGT

SEQ ID NO: 4 - protein, 4 aa, unidentified
WNIP

SEQ ID NO: 5 - protein, 9 aa, unidentified
AGWNIPIGT

SEQ ID NO: 6 - protein, 7 aa, unidentified
RADHPFL

SEQ ID NO: 7 - protein, 8 aa, unidentified
FPFEVFGK

SEQ ID NO: 8 - protein, 7 aa, unidentified
FGRCVSP

SEQ ID NO: 9 - protein, 8 aa, unidentified
FFGRCVSP